European Patent Application EP 4 790 069 A1, published August 12, 2026. Title: ヒトＣＤ１５３を標的とする抗体ならびにキメラ抗原受容体. Applicant: 国立大学法人京都大学. The sequence listing filed with the application follows.

SEQUENCE LISTING (16 sequences)

SEQ ID NO: 1 - protein, 5 aa, Mus musculus
NYWLG

SEQ ID NO: 2 - protein, 17 aa, Mus musculus
DIYPGNYNSYSNEKFKG

SEQ ID NO: 3 - protein, 10 aa, Mus musculus
IYGNYWIFDV

SEQ ID NO: 4 - protein, 10 aa, Mus musculus
SASSSVNYMH

SEQ ID NO: 5 - protein, 7 aa, Mus musculus
STSDLAS

SEQ ID NO: 6 - protein, 9 aa, Mus musculus
QQRSSYPLT

SEQ ID NO: 7 - protein, 151 aa, Mus musculus
MSSPQTLNTLTLTMGWSWIFLFLLSGTAGVLSEVQLQQSGPELVKPGASVKISCKASGYTFTDYYMNWVKQSHGKTLEWIGDINPNHGGATYNQKFKGKATLTVDKSSSTAYMELRSLTSEDSAVYYCASPYDGYYGFAYWGQGTLVTVSA

SEQ ID NO: 8 - protein, 127 aa, Mus musculus
MVSTPQFLVFLLFWIPASRGDILLTQSPAILSVSPGERVSFSCRASQSIGTSIHWYQQRTNGSPRLLIKYGSESISGIPSRFSGSGSGTDFTLSINSVESEDIADYYCQQSNSWPTTFGGGTKLEIK

SEQ ID NO: 9 - protein, 5 aa, Mus musculus
DYYMN

SEQ ID NO: 10 - protein, 17 aa, Mus musculus
DINPNHGGATYNQKFKG

SEQ ID NO: 11 - protein, 10 aa, Mus musculus
PYDGYYGFAY

SEQ ID NO: 12 - protein, 11 aa, Mus musculus
RASQSIGTSIH

SEQ ID NO: 13 - protein, 7 aa, Mus musculus
YGSESIS

SEQ ID NO: 14 - protein, 9 aa, Mus musculus
QQSNSWPTT

SEQ ID NO: 15 - protein, 138 aa, Mus musculus
MEWSGVFIFLLSVSTGVHSRVQLQQSGAELVRPGTSVKISCKASGYAFTNYWLGWVKQRPGHGLEWIGDIYPGNYNSYSNEKFKGKATLTADESSSTAYMQLSSLTSEDSAVYFCARIYGNYWIFDVWGAGTTVTVSS

SEQ ID NO: 16 - protein, 128 aa, Mus musculus
MHFQVQIFSFLLISASVIMSRGQIVLTQSPAIMSASPGEKVTMTCSASSSVNYMHWFQQKPGTSPKLWIYSTSDLASGVPARFSGSGSGTSYSLTISRMEAEDAATYYCQQRSSYPLTFGAGTKLELK